European Patent Specification EP 4 499 869 B1, published July 15, 2026. Title: Primers and probes for detecting mycobacteria. Applicant: Sanofi Pasteur. Application EP. The sequence listing filed with the application follows.

SEQUENCE LISTING (39 sequences)

SEQ ID NO: 1 - DNA, 20 bp, synthetic construct
  misc_feature 1..20: note = primer
  source 1..20: mol_type = other DNA
cctggtagtccacgccgtaa

SEQ ID NO: 2 - DNA, 20 bp, synthetic construct
  misc_feature 1..20: note = primer
  source 1..20: mol_type = other DNA
cggatcccaaggaaggaaac

SEQ ID NO: 3 - DNA, 18 bp, synthetic construct
  misc_feature 1..18: note = probe
  source 1..18: mol_type = other DNA
cggtgggtactaggtgtg

SEQ ID NO: 4 - DNA, 20 bp, synthetic construct
  misc_feature 1..20: note = primer
  source 1..20: mol_type = other DNA
cacaggacgccggtagagat

SEQ ID NO: 5 - DNA, 19 bp, synthetic construct
  misc_feature 1..19: note = Primer
  source 1..19: mol_type = other DNA
catgcaccacctgcacaca

SEQ ID NO: 6 - DNA, 16 bp, synthetic construct
  misc_feature 1..16: note = probe
  source 1..16: mol_type = other DNA
tcggttcccttgtggc

SEQ ID NO: 7 - DNA, 20 bp, synthetic construct
  misc_feature 1..20: note = primer
  source 1..20: mol_type = other DNA
cccttatgtccagggcttca

SEQ ID NO: 8 - DNA, 17 bp, synthetic construct
  misc_feature 1..17: note = primer
  source 1..17: mol_type = other DNA
ggcatcgcagccctttg

SEQ ID NO: 9 - DNA, 18 bp, synthetic construct
  misc_feature 1..18: note = probe
  source 1..18: mol_type = other DNA
acatgctacaatggccgg

SEQ ID NO: 10 - DNA, 21 bp, synthetic construct
  misc_feature 1..21: note = primer
  source 1..21: mol_type = other DNA
cctggtagtccacgccgtaaa

SEQ ID NO: 11 - DNA, 20 bp, synthetic construct
  misc_feature 1..20: note = primer
  source 1..20: mol_type = other DNA
ctggtagtccacgccgtaaa

SEQ ID NO: 12 - DNA, 21 bp, synthetic construct
  misc_feature 1..21: note = primer
  source 1..21: mol_type = other DNA
acggatcccaaggaaggaaac

SEQ ID NO: 13 - DNA, 20 bp, synthetic construct
  misc_feature 1..20: note = primer
  source 1..20: mol_type = other DNA
ggatcccaaggaaggaaacc

SEQ ID NO: 14 - DNA, 21 bp, synthetic construct
  misc_feature 1..21: note = primer
  source 1..21: mol_type = other DNA
cacaggacgccggtagagata

SEQ ID NO: 15 - DNA, 20 bp, synthetic construct
  misc_feature 1..20: note = primer
  source 1..20: mol_type = other DNA
catgcaccacctgcacacag

SEQ ID NO: 16 - DNA, 19 bp, synthetic construct
  misc_feature 1..19: note = primer
  source 1..19: mol_type = other DNA
atgcaccacctgcacacag

SEQ ID NO: 17 - DNA, 18 bp, synthetic construct
  misc_feature 1..18: note = primer
  source 1..18: mol_type = other DNA
tgcaccacctgcacacag

SEQ ID NO: 18 - DNA, 20 bp, synthetic construct
  misc_feature 1..20: note = primer
  source 1..20: mol_type = other DNA
ccccttatgtccagggcttc

SEQ ID NO: 19 - DNA, 18 bp, synthetic construct
  misc_feature 1..18: note = primer
  source 1..18: mol_type = other DNA
gccccttatgtccagggc

SEQ ID NO: 20 - DNA, 16 bp, synthetic construct
  misc_feature 1..16: note = primer
  source 1..16: mol_type = other DNA
cggcatcgcagccctt

SEQ ID NO: 21 - DNA, 19 bp, synthetic construct
  misc_feature 1..19: note = primer
  source 1..19: mol_type = other DNA
ggcatcgcagccctttgta

SEQ ID NO: 22 - DNA, 17 bp, synthetic construct
  misc_feature 1..17: note = probe
  source 1..17: mol_type = other DNA
cggtgggtactaggtgt

SEQ ID NO: 23 - DNA, 16 bp, synthetic construct
  misc_feature 1..16: note = probe
  source 1..16: mol_type = other DNA
cggtgggtactaggtg

SEQ ID NO: 24 - DNA, 17 bp, synthetic construct
  misc_feature 1..17: note = probe
  source 1..17: mol_type = other DNA
atcggttcccttgtggc

SEQ ID NO: 25 - DNA, 15 bp, synthetic construct
  misc_feature 1..15: note = probe
  source 1..15: mol_type = other DNA
cggttcccttgtggc

SEQ ID NO: 26 - DNA, 19 bp, synthetic construct
  misc_feature 1..19: note = probe
  source 1..19: mol_type = other DNA
acatgctacaatggccggt

SEQ ID NO: 27 - DNA, 22 bp, synthetic construct
  misc_feature 1..22: note = primer
  source 1..22: mol_type = other DNA
cacggatcccaaggaaggaaac

SEQ ID NO: 28 - DNA, 18 bp, synthetic construct
  misc_feature 1..18: note = primer
  source 1..18: mol_type = other DNA
gcatcgcagccctttgta

SEQ ID NO: 29 - DNA, 19 bp, synthetic construct
  misc_feature 1..19: note = Primer
  source 1..19: mol_type = other DNA
tggtagtccacgccgtaaa

SEQ ID NO: 30 - DNA, 22 bp, synthetic construct
  misc_feature 1..22: note = Primer
  source 1..22: mol_type = other DNA
gcacggatcccaaggaaggaaa

SEQ ID NO: 31 - DNA, 22 bp, synthetic construct
  misc_feature 1..22: note = Primer
  source 1..22: mol_type = other DNA
acggatcccaaggaaggaaacc

SEQ ID NO: 32 - DNA, 20 bp, synthetic construct
  misc_feature 1..20: note = Primer
  source 1..20: mol_type = other DNA
acaggacgccggtagagata

SEQ ID NO: 33 - DNA, 19 bp, synthetic construct
  misc_feature 1..19: note = Primer
  source 1..19: mol_type = other DNA
caggacgccggtagagata

SEQ ID NO: 34 - DNA, 21 bp, synthetic construct
  misc_feature 1..21: note = primer
  source 1..21: mol_type = other DNA
ccccttatgtccagggcttca

SEQ ID NO: 35 - DNA, 21 bp, synthetic construct
  misc_feature 1..21: note = primer
  source 1..21: mol_type = other DNA
gccccttatgtccagggcttc

SEQ ID NO: 36 - DNA, 17 bp, synthetic construct
  misc_feature 1..17: note = Primer
  source 1..17: mol_type = other DNA
cggcatcgcagcccttt

SEQ ID NO: 37 - DNA, 17 bp, synthetic construct
  misc_feature 1..17: note = Primer
  source 1..17: mol_type = other DNA
gcatcgcagccctttgt

SEQ ID NO: 38 - DNA, 17 bp, synthetic construct
  misc_feature 1..17: note = probe
  source 1..17: mol_type = other DNA
catgctacaatggccgg

SEQ ID NO: 39 - DNA, 16 bp, synthetic construct
  misc_feature 1..16: note = Probe
  source 1..16: mol_type = other DNA
catgctacaatggccg